European Patent Application EP 4 253 557 A1, published October 4, 2023. Title: PRIMER AND PROBE DESIGN METHOD, DETECTION COMPOSITION, AND KIT FOR MIRNA DETECTION. Applicant: SANSURE BIOTECH INC. The sequence listing filed with the application follows.

SEQUENCE LISTING (56 sequences)

SEQ ID NO: 1 - DNA, 44 bp, Artificial sequence
gtcgtatccagtgcagggtccgaggtattcgcactggatacgac

SEQ ID NO: 2 - DNA, 48 bp, Artificial sequence
gtcgtatccagtgcgtgtcgtggagtcggcaattgcactggatacgac

SEQ ID NO: 3 - DNA, 36 bp, Artificial sequence
gatgaggagtgtcgtggagtcggcaatttcctcatc

SEQ ID NO: 4 - DNA, 37 bp, Artificial sequence
ctcaactggtgtcgtggagtcggcaattcagttgagc

SEQ ID NO: 5 - RNA, 23 nt, homo sapiens
aaaagugcuuacagugcagguag

SEQ ID NO: 6 - RNA, 22 nt, homo sapiens
ugagguaguagguuguauaguu

SEQ ID NO: 7 - RNA, 21 nt, homo sapiens
uucaaguaauucaggauaggu

SEQ ID NO: 8 - RNA, 22 nt, homo sapiens
uauugcacuugucccggccugu

SEQ ID NO: 9 - DNA, 22 bp, Artificial sequence
gcgtcaaaagtgcttacagtgc

SEQ ID NO: 10 - DNA, 20 bp, Artificial sequence
gtagcgtggagtcggcaatt

SEQ ID NO: 11 - DNA, 18 bp, Artificial sequence
atcggatacgacctacct

SEQ ID NO: 12 - DNA, 52 bp, Artificial sequence
gtcgtatccgatcgtagcgtggagtcggcaattgatcggatacgacctacct

SEQ ID NO: 13 - DNA, 21 bp, Artificial sequence
gcggctgaggtagtaggttgt

SEQ ID NO: 14 - DNA, 19 bp, Artificial sequence
gaaggctggagagcgagat

SEQ ID NO: 15 - DNA, 18 bp, Artificial sequence
tacgactacgataactat

SEQ ID NO: 16 - DNA, 51 bp, Artificial sequence
atcgtagtcgtacgaaggctggagagcgagatgtacgactacgataactat

SEQ ID NO: 17 - DNA, 21 bp, Artificial sequence
tcgccattcaagtaattcagg

SEQ ID NO: 18 - DNA, 19 bp, Artificial sequence
ctcacgctcgagacggatc

SEQ ID NO: 19 - DNA, 19 bp, Artificial sequence
cgagcaatagctcacctat

SEQ ID NO: 20 - DNA, 55 bp, Artificial sequence
gagctattgctcgcctcacgctcgagacggatctggcgagcaatagctcacctat

SEQ ID NO: 21 - DNA, 19 bp, Artificial sequence
cgctattgcacttgtcccg

SEQ ID NO: 22 - DNA, 20 bp, Artificial sequence
cgagagctgctcacggagat

SEQ ID NO: 23 - DNA, 18 bp, Artificial sequence
catcctcatgctacaggc

SEQ ID NO: 24 - DNA, 51 bp, Artificial sequence
agcatgaggatgcgagagctgctcacggagatgcatcctcatgctacaggc

SEQ ID NO: 25 - DNA, 23 bp, Artificial sequence
gccgagaaaagtgcttacagtgc

SEQ ID NO: 26 - DNA, 20 bp, Artificial sequence
gtgtcgtggagtcggcaatt

SEQ ID NO: 27 - DNA, 19 bp, Artificial sequence
cactggatacgacctacct

SEQ ID NO: 28 - DNA, 54 bp, Artificial sequence
gtcgtatccagtgcgtgtcgtggagtcggcaattgcactggatacgacctacct

SEQ ID NO: 29 - DNA, 23 bp, Artificial sequence
cggcaggtgaggtagtaggttgt

SEQ ID NO: 30 - DNA, 21 bp, Artificial sequence
agtgcagggtccgaggtattc

SEQ ID NO: 31 - DNA, 18 bp, Artificial sequence
actggatacgacaactat

SEQ ID NO: 32 - DNA, 50 bp, Artificial sequence
gtcgtatccagtgcagggtccgaggtattcgcactggatacgacaactat

SEQ ID NO: 33 - DNA, 21 bp, Artificial sequence
ccgccattcaagtaattcagg

SEQ ID NO: 34 - DNA, 21 bp, Artificial sequence
agtgcagggtccgaggtattc

SEQ ID NO: 35 - DNA, 19 bp, Artificial sequence
cactggatacgacacctat

SEQ ID NO: 36 - DNA, 50 bp, Artificial sequence
gtcgtatccagtgcagggtccgaggtattcgcactggatacgacacctat

SEQ ID NO: 37 - DNA, 19 bp, Artificial sequence
ccgtattgcacttgtcccg

SEQ ID NO: 38 - DNA, 20 bp, Artificial sequence
gtgtcgtggagtcggcaatt

SEQ ID NO: 39 - DNA, 18 bp, Artificial sequence
actggatacgacacaggc

SEQ ID NO: 40 - DNA, 54 bp, Artificial sequence
gtcgtatccagtgcgtgtcgtggagtcggcaattgcactggatacgacacaggc

SEQ ID NO: 41 - DNA, 21 bp, Artificial sequence
tatccgatcgtagcgtggagt

SEQ ID NO: 42 - DNA, 19 bp, Artificial sequence
cgatcgtagcgtggagtcg

SEQ ID NO: 43 - DNA, 20 bp, Artificial sequence
cgtggagtcggcaattgatc

SEQ ID NO: 44 - DNA, 22 bp, Artificial sequence
gcgtcaaaagtgcttacagtgc

SEQ ID NO: 45 - DNA, 20 bp, Artificial sequence
gtagcgtggagtcggcaatt

SEQ ID NO: 46 - DNA, 18 bp, Artificial sequence
atcggatacgacctacct

SEQ ID NO: 47 - DNA, 52 bp, Artificial sequence; identical to SEQ ID NO: 12

SEQ ID NO: 48 - DNA, 22 bp, Artificial sequence
cgtcaaaagtgcttacagtgca

SEQ ID NO: 49 - DNA, 17 bp, Artificial sequence
atcggatacgacctacc

SEQ ID NO: 50 - DNA, 51 bp, Artificial sequence
gtcgtatccgatcgtagcgtggagtcggcaattgatcggatacgacctacc

SEQ ID NO: 51 - DNA, 22 bp, Artificial sequence
ggcgtcaaaagtgcttacagtg

SEQ ID NO: 52 - DNA, 19 bp, Artificial sequence
atcggatacgacctacctg

SEQ ID NO: 53 - DNA, 53 bp, Artificial sequence
gtcgtatccgatcgtagcgtggagtcggcaattgatcggatacgacctacctg

SEQ ID NO: 54 - DNA, 22 bp, Artificial sequence
cggcgtcaaaagtgcttacagt

SEQ ID NO: 55 - DNA, 21 bp, Artificial sequence
atcggatacgacctacctgca

SEQ ID NO: 56 - DNA, 55 bp, Artificial sequence
gtcgtatccgatcgtagcgtggagtcggcaattgatcggatacgacctacctgca